European Patent Specification EP 3 430 042 B1, published May 24, 2023. Title: Anti-TNF-alpha antibodies and functional fragments thereof. Applicant: Numab Innovation AG. The sequence listing filed with the application follows.

SEQUENCE LISTING (27 sequences)

SEQ ID NO: 1 - protein, 12 aa, Artificial Sequence
  CDR L1 of clones 16-02-B03, 16-04-F06 and 16-23-C06
QSSQSVYSSNLA

SEQ ID NO: 2 - protein, 7 aa, Artificial Sequence
  CDR L2 of clones 16-02-B03, 16-04-F06 and 16-23-C06
SASKLAS

SEQ ID NO: 3 - protein, 12 aa, Artificial Sequence
  CDR L3 of clones 16-02-B03, 16-04-F06 and 16-23-C06
QGTYYTSNWLNA

SEQ ID NO: 4 - protein, 10 aa, Artificial Sequence
  CDR H1 of clones 16-02-B03, 16-04-F06 and 16-23-C06
GIDLSSYAMG

SEQ ID NO: 5 - protein, 16 aa, Artificial Sequence
  Generic CDR H2
  MISC_FEATURE (4)..(4): Xaa is Val or Ile
  MISC_FEATURE (7)..(7): Xaa is Ser or Asn
TISXGGXTYYANWAEG

SEQ ID NO: 6 - protein, 11 aa, Artificial Sequence
  CDR H3 of clones 16-02-B03, 16-04-F06 and 16-23-C06
GDYINFFYFNI

SEQ ID NO: 7 - protein, 16 aa, Artificial Sequence
  CDR H2 of clone 16-02-B03
TISVGGSTYYANWAEG

SEQ ID NO: 8 - protein, 16 aa, Artificial Sequence
  CDR H2 of clone 16-04-F06
TISIGGSTYYANWAEG

SEQ ID NO: 9 - protein, 16 aa, Artificial Sequence
  CDR H2 of clone 16-23-C06
TISIGGNTYYANWAEG

SEQ ID NO: 10 - protein, 112 aa, Artificial Sequence
  VL of humanized scFv of clone 16-02-B03-sc02
DIQMTQSPSSLSASVGDRVTITCQSSQSVYSSNLAWYQQKPGKAPKLLIYSASKLASGVPSRFSGSGSGTDFTLTISSLQPEDEATYYCQGTYYTSNWLNAFGGGTKLTVLG

SEQ ID NO: 11 - protein, 119 aa, Artificial Sequence
  VH of humanized scFv of clone 16-02-B03-sc02
EVQLVESGGGLVQPGGSLRLSCAASGIDLSSYAMGWVRQAPGKGLEWIGTISVGGSTYYANWAEGRFTISRDNSKNTVYLQMNSLRAEDTAVYYCAGGDYINFFYFNIWGQGTLVTVSS

SEQ ID NO: 12 - protein, 252 aa, Artificial Sequence
  Humanized scFv of clone 16-02-B03-sc02
MDIQMTQSPSSLSASVGDRVTITCQSSQSVYSSNLAWYQQKPGKAPKLLIYSASKLASGVPSRFSGSGSGTDFTLTISSLQPEDEATYYCQGTYYTSNWLNAFGGGTKLTVLGGGGGSGGGGSGGGGSGGGGSEVQLVESGGGLVQPGGSLRLSCAASGIDLSSYAMGWVRQAPGKGLEWIGTISVGGSTYYANWAEGRFTISRDNSKNTVYLQMNSLRAEDTAVYYCAGGDYINFFYFNIWGQGTLVTVSS

SEQ ID NO: 13 - protein, 112 aa, Artificial Sequence
  VL of humanized scFv of clone 16-02-B03-sc05
DIQMTQSPSSLSASVGDRVTINCQSSQSVYSSNLAWYQQKPGKAPKLLIYSASKLASGVPSRFSGSGSGTQFTLTISGLQPDDFATYYCQGTYYTSNWLNAFGGGTKLTVLG

SEQ ID NO: 14 - protein, 119 aa, Artificial Sequence
  VH of humanized scFv of clone 16-02-B03-sc05
EVQLVESGGGLVQPGGSLRLSCTASGIDLSSYAMGWVRQAPGKGLEWIGTISVGGSTYYANWAEGRFTISKDTSKNTVYLQMNSLRAEDTAVYYCAGGDYINFFYFNIWGQGTLVTVSS

SEQ ID NO: 15 - protein, 252 aa, Artificial Sequence
  Humanized scFv of clone 16-02-B03-sc05
MDIQMTQSPSSLSASVGDRVTINCQSSQSVYSSNLAWYQQKPGKAPKLLIYSASKLASGVPSRFSGSGSGTQFTLTISGLQPDDFATYYCQGTYYTSNWLNAFGGGTKLTVLGGGGGSGGGGSGGGGSGGGGSEVQLVESGGGLVQPGGSLRLSCTASGIDLSSYAMGWVRQAPGKGLEWIGTISVGGSTYYANWAEGRFTISKDTSKNTVYLQMNSLRAEDTAVYYCAGGDYINFFYFNIWGQGTLVTVSS

SEQ ID NO: 16 - protein, 112 aa, Artificial Sequence
  VL of humanized scFv of clone 16-02-B03-sc06
DIQMTQSPSSLSASVGDRVTITCQSSQSVYSSNLAWYQQKPGKAPKLLIYSASKLASGVPSRFSGSGSGTDFTLTISSLQPEDEATYYCQGTYYTSNWLNAFGCGTKLTVLG

SEQ ID NO: 17 - protein, 119 aa, Artificial Sequence
  VH of humanized scFv of clone 16-02-B03-sc06
EVQLVESGGGLVQPGGSLRLSCAASGIDLSSYAMGWVRQAPGKCLEWIGTISVGGSTYYANWAEGRFTISRDNSKNTVYLQMNSLRAEDTAVYYCAGGDYINFFYFNIWGQGTLVTVSS

SEQ ID NO: 18 - protein, 252 aa, Artificial Sequence
  Humanized scFv of clone 16-02-B03-sc06
MDIQMTQSPSSLSASVGDRVTITCQSSQSVYSSNLAWYQQKPGKAPKLLIYSASKLASGVPSRFSGSGSGTDFTLTISSLQPEDEATYYCQGTYYTSNWLNAFGCGTKLTVLGGGGGSGGGGSGGGGSGGGGSEVQLVESGGGLVQPGGSLRLSCAASGIDLSSYAMGWVRQAPGKCLEWIGTISVGGSTYYANWAEGRFTISRDNSKNTVYLQMNSLRAEDTAVYYCAGGDYINFFYFNIWGQGTLVTVSS

SEQ ID NO: 19 - protein, 20 aa, Artificial Sequence
  Linker sequence in scFv
GGGGSGGGGSGGGGSGGGGS

SEQ ID NO: 20 - protein, 5 aa, Artificial Sequence
  Linker sequence in diabody
GGGGS

SEQ ID NO: 21 - protein, 23 aa, Artificial Sequence
  Vk1 consensus sequences framework I
DIQMTQSPSSLSASVGDRVTITC

SEQ ID NO: 22 - protein, 15 aa, Artificial Sequence
  Vk1 consensus sequence framework II
WYQQKPGKAPKLLIY

SEQ ID NO: 23 - protein, 32 aa, Artificial Sequence
  Vk1 consensus sequence framework III
GVPSRFSGSGSGTDFTLTISSLQPEDFATYYC

SEQ ID NO: 24 - protein, 10 aa, Artificial Sequence
  V lambda  germline-based framework IV sequence
FGTGTKVTVL

SEQ ID NO: 25 - protein, 10 aa, Artificial Sequence
  V lambda  germline-based framework IV sequence
FGGGTKLTVL

SEQ ID NO: 26 - protein, 10 aa, Artificial Sequence
  V lambda  germline-based framework IV sequence
FGGGTQLIIL

SEQ ID NO: 27 - protein, 10 aa, Artificial Sequence
  V lambda  germline-based framework IV sequence
FGSGTKVTVL